European Patent Application EP 4 206 326 A1, published July 5, 2023. Title: An enzyme dehydroxylating the hydroxyl group at the 9-position of a urolithin. Applicant: Daicel Corporation. The sequence listing filed with the application follows.

SEQUENCE LISTING (24 sequences)

SEQ ID NO: 1 - protein, 289 aa, Clostridium bolteae
MVLPQFEYLAPKTIGEACNLFLELGSTARVMAGATDLIPPMKDKVISPEYIIDLKKIPGLDYLEYDDREGLKIGALTTLRTIETSPLVKEKNPAVAHAAKVVASTQIRTKGTMAGNICNASPSCDTAPNLLAQGAKILVQGPNKDRVIQIEDFFLGVKKTSLEPGEIVTGIVIPPLAENERAAYIKHAVRKAMDLAIIGVAVKIKVEDGVCTDARIALGAVAATPVRAPGAEEALIGKELTDEVIVKASEEAMNSCHPISDIRASAEYRKDMIRVFTKRAIKQAMECYN

SEQ ID NO: 2 - protein, 163 aa, Clostridium bolteae
MKHSISLIINGDPVDAIVKDNLTLLDFLRDQLFLTGTKKGCEEGECGACTVMLDGKPVNSCCTLAVECDGHEIITVEGIAREGMLHPIQKQFIEKWAMQCGYCTPGMIMSAKALLDVNKHPTELEIREAIEGNLCRCTGYAKIVEAIQAAAAQMNWEEEAKNA

SEQ ID NO: 3 - protein, 787 aa, Clostridium bolteae
MHKDCDKHYFKKPEFYRLTGENNYVRIDAEDKVTGHGQYVGDIMFPDMLTGKMVRSPYASAKILSIDTSEAEKLPGVKCILTARDFEWKSLVGNGEFAAEFADKEVLCSEKVRQVGDDVAAVAAVDEETAQRAADLIKVEYQVLPGVFDPFEAMEENAPEVNWEGKGIHNIGMQSVMKAGTDIDEEFDRASYVQHRDYKTHRMVHAAMEPHGAVATYRNGTYTIWMSTQMSFVDQFWYARCLGVGENQVRVIKPLVGGGFGGKLDSYSFGLCAAKMAEMTGRPVRMILSREEVFQTTRNRHPIYMHIDTAFGTDGKLLAKKCYHVLDGGPYGGSGVAACAQSTLWANFPYKMNSVDFLARRVYTNNPSAGAMRGYTACQVHFAHDLNMQFAADQMGIDPVEFRKISAADPGYVAPAGLAITSCAYKETLDTAAKEIGWYEKKDKLKKGEGIGFAGTGFVSGTGFAVLEAPNQSSACVTLRMNKRGMATLYIGSHDIGQGSDTVMTAIVAEELGLPMDMVKTFMSDTFLTPWDSGSYGSRVTFLAGNAARRAAVDAKRQLFEVIAPMWGVMPETLECLDGKVISKEKAEYQMSIGDAMFKYMTVKGGDELIGVGSYYHRTDNSQYNGNNTTNYAPAYSFSTGAAHLTVDEETGVLDIDEFVFAHDCGRALNKRAVEGQLEGSIGMGLGYAVYEHNVTREGKILNPNFRDYRLPTALDMPKMRTFYDFTPDEEGPLGAKEAGEGSAAPVAPAIANAVNMATGVYFTELPLDPEHIWRALHGMKDDRNSK

SEQ ID NO: 4 - protein, 288 aa, Clostridium asparagiforme
MVLPQFEYLAPKTIGEACNLLLELGSTAKVMAGATDLIPPMKDKVIAPEYIIDLKKIPGLDDLEYDEKEGLKIGALTTLRAIETSPLVKEKNPAIAHAAKVVASTQIRAKGTMAGNICNASPSCDTAPNLLAQGAKILVQGPNKDRVIKIDDFFLGVKKTSLEPGEIVTGIVIPPLAENERAAYIKHAVRKAMDLAIIGVAVKIRVEVGICTDAKIALGAVAATPIRAPRAEEALIGKALTDEVIVRASEEAMNSCHPISDIRASAEYRKDMIRVFTKRAIKQAMESL

SEQ ID NO: 5 - protein, 163 aa, Clostridium asparagiforme
MKHSISLIINGDPVDAIVKDNLTLLDFLRDQMFLTGTKKGCEEGECGACTVMLDGKPVNSCCTLAVECDGHEILTVEGVAKEGMLHPIQKQFIEKWAMQCGYCTPGMIMSAKALLDVNRHPTELEIREAIEGNLCRCTGYAKIVEAIQAAADEMNWEEESENA

SEQ ID NO: 6 - protein, 787 aa, Clostridium asparagiforme
MHKDCDKHYFKKPEFYRLTGGNNYVRIDAEDKVTGHGQYVGDIMFPDMLTGKMVRSPYASARIISIDTSAAEKLPGVKCILTAKDFEWKSLVGNGEFAAEFADKEVLCSEKVRQVGDDIAAVAAVDEETAQRAVDLIKVEYEVLPGVFDPFEAMEDDAPEVNWEGKGIHNIGMQSVMKAGTDIDQEFDSASYVQHRDYKTHRMVHAAMEPHGAVATYRNGTYTIWMSTQMSFVDQFWYARCLGVGENQVRVIKPLVGGGFGGKLDSYSFGLCAAKMSEITGRPVRMILSREEVFQTTRNRHPIYMHIDTAFGADGRLLAKKCYHVLDGGPYGGSGVAACAQSTLWANFPYKMNSVDFLARRVYTNNPSAGAMRGYTACQVHFAHDLNMQFAADQLGMDPVEFRKISAADPGYVAPAGLAITSCAYKETLDTAAREIGWNEKKDKMKKGEGIGFAGTGFVSGTGFAVLEAPNQSSACVTLRMNKRGMATLYIGSHDIGQGSDTVMTAIVAEELGLPMNMVKTFMSDTFLTPWDSGSYGSRVTFLAGNAARRAAVDAKRQLFEVIAPMWGVMPETLECLDGKVISRENAQLQMPIGDAMFKYMTVKGGDELIGVGSYYHRTDNSQYNGTNTTNYAPAYSFSTGAAHLTVDEETGVLDIDEFVFAHDCGRALNKRAVEGQLEGSIGMGLGYAVYEHNVTKEGKILNPNFRDYRLPTALDMPKMRTFYDFTPDEEGPLGAKEAGEGSAAPVAPAIANAVNMATGVYFTELPLDPEHIWRALHGMKDDRNSK

SEQ ID NO: 7 - protein, 288 aa, Clostridium citroniae
MVLPQFEYLAPKTIGEACNLLLELGSPAKVMAGATDLIPPMKDKAISPEYLIDLKKIPDLDYLEYDEKEGLKIGALTTLRTIETSPLVKEKNPAVAHAAKVVASTQIRAKGTMAGNICNASPSCDTAPNLLAQGAKILVQGPNKDRIIQAEDFFLGVKKTSLEPGEIVTGIVIPPLAENERAAYIKHAVRKAMDLAIIGVAVKIKVEDGICTDVHIALGAVAATPIRAPKAEEALIGKALTDEVIVKASEEAMDSCHPISDIRASAEYRKDMIRVFTKRAVRQAMECL

SEQ ID NO: 8 - protein, 163 aa, Clostridium citroniae
MKHSISLTVNGDCVDAVVKDNLTLLDFLRDQLFLTGTKKGCEEGECGACTVMLDGKPVNSCCTLAVECDGHDIITVEGIAENGMLHPIQKQFIEKWAMQCGYCTPGMIMSAKALLDVNRHPTELEIREAIEGNLCRCTGYAKIVEAIQAAAAQMNWEEESENA

SEQ ID NO: 9 - protein, 787 aa, Clostridium citroniae
MHKDCDKHYFKKPEFYRLTGENHYVRIDAEDKVTGHGQYVGDIMFPDMLTGKMVRSPYASARILSIDTSEAEKLPGVKCILTAKDFEWKSLVGNGEFAAEFADKEVLCSEKVRQVGDDVAAVAAVDEETAQRAVDLIKVEYEVLPGVFDPFEAMEEGAPEVNWEGKGLHNIGMQSVMKAGTDIDQEFDNAGYVQHRDYKTHRMVHAAMEPHGAVATFRNGTYTIWMSTQMSYVDQFWYARCLGVGENQVRVIKPLVGGGFGGKLDSYSFGLCAAKMSELTGRPVRMILSREEVFQTTRNRHPIYMHIDTAFGADGKLLAKKCYHVLDGGPYGGSGVAACAQSTLWANFPYKMNSVDFLARRVYTNNPSAGAMRGYTACQVHFAHDLNMQFAADQMGIDPVEFRKMSAADPGYVAPAGLAITSCAYKETLDTAAREIGWYDKKDQMKKGEGIGFAGTGFVSGTGFAVLEAPNQSSACVTLRMNKRGMATLYIGSHDIGQGSDTVMTAIVAEELGLPMDMVKTFMSDTFLTPWDSGSYGSRVTFLAGNAARRAAVDAKRQLFEVIAPMWGVMPETLECLDGKVISKENAELQMPIGDAMFKYMTVKGGDELVGIGSYYHRTDNSQYNGTNTTNYAPAYSFSTGAAHLTVDEETGVLDIDEFVFAHDCGRALNKRAVEGQLEGSIGMGLGYAVYEHNVTKEGKILNPNFRDYRLPTALDMPKMRTFYDFTPDEEGPLGAKEAGEGSAAPVAPAIANAVNMATGVYFTELPLDPEHIWRALHGLKDDRNSK

SEQ ID NO: 10 - DNA, 870 bp, Clostridium bolteae
ctagttatagcattccatggcctgcttaatggcacgttttgtaaacacgcggatcatatccttcctgtattcggccgatgcgcggatatcagagattggatgacaggaattcattgcttcctccgatgccttcacaatcacttcatcggtaagttctttgccaatcagggcttcctccgccccgggtgcccgtaccggcgtggccgcaaccgcgcccagggcaatcctggcgtctgtgcagacgccgtcttccaccttaatcttgactgcgacgccgatgatggccaggtccatcgcctttctgaccgcgtgttttatgtatgcagccctctcattctcagccagcggcggaatcacaatgcctgtcacgatttctcccggctccagggaagtctttttgacacccaggaaaaagtcttcgatttgaatgacccggtccttgttgggaccctgtaccaatatcttagcgccctgagccagtaggttgggggctgtatcgcaggatggggacgcattgcagatattgcctgccatggtgccctttgtcctgatttgtgtggatgccactaccttggcggcatgagccactgccggattcttttctttaaccagaggagatgtctctatggtacgcagtgttgtcagcgcccctatttttaaaccttccctgtcatcgtattccagataatccaaacctggaattttcttaaggtcaatgatatactctggtgatataaccttgtctttcattggcggaatcagatccgttgcgcctgccataaccctggctgtgcttccaagctcaaggaacagattgcacgcctccccgatggtcttaggagcaagatactcgaattgaggtaataccat

SEQ ID NO: 11 - DNA, 492 bp, Clostridium bolteae
ttatgcattctttgcttcctcctcccagttcatctgcgcagcggctgcctggattgcctccacaatctttgcataaccggtgcagcggcacagattgccctcaatggcttcccggatttccagttccgtaggatgtttattcacatccagaagagctttggcggacataatcatacccggagtacagtagccgcactgcatggcccacttctctataaactgcttctgaatgggatgaagcatcccctccctggcaattccctccacggttatgatctcatggccgtcgcactccacggccagggtacagcaggagttaaccggcttaccgtcaagcatcacggtacaggcgccacactccccttcctcacacccctttttcgtgcctgtcagaaacaactggtcacgaagaaaatccagaagcgtcaggttatccttcacaatagcatcaaccggatctccgttgatgattaaacttatactatgtttcat

SEQ ID NO: 12 - DNA, 2364 bp, Clostridium bolteae
ttattttgaattcctgtcatccttcatgccgtgcagcgctctccagatatgctccgggtccagaggcagctctgtgaagtacacgccggttgccatgttgaccgcattggcaatggcaggcgccacaggtgctgcggagccctcgccagcttcctttgcgcccagaggtccttcctcgtccggtgtaaagtcgtaaaaggtgcgcatcttcggcatatcaagggcagtgggcagccggtaatcgcggaagttgggattgagaatctttccttccctggttacattgtgctcatagacagcatagcccaggcccatgccgatggatccctccagctggccttccacggccctcttattcagtgcgcggccgcagtcatgggcaaatacaaattcatcaatatccaggacgccggtctcctcgtccacagtcagatgggctgctccggtggagaagctgtatgcaggcgcgtagttggtggtattgttgccgttatactgtgaattgtcggtacggtggtaataggatcccacgccaatcagttcatcgccgcccttgaccgtcatatacttgaacatggcgtctccaatggacatctgatactctgccttctccttgctgattacctttccgtccagacactctaatgtctccggcatcaccccccacataggcgcaatgacctcaaacagctggcgttttgcatccacggcagcgcggcgggccgcattgccggccaggaaggtaacacggctgccgtaagagccggagtcccagggcgtcaggaaggtgtcggacataaaggtcttgaccatatccatgggaagccccagttcctcggccacaatggccgtcataaccgtatcggaaccctgtcctatgtcgtgggagccgatgtacagggtggccatgccccgcttgttcatgcgcagggtcacgcacgcagagctctggttgggcgcttccagcaccgcgaatccggtgcccgatacaaagccggtgcccgcaaaaccaatgccctctccctttttcagcttatccttcttctcataccagccaatttcctttgcagccgtatccagtgtctccttgtatgcgcagctggtgattgccagtccggccggagccacgtatccggggtctgccgcgcttatcttgcggaactcaaccgggtcaatgcccatctggtcagccgcgaactgcatgttcaggtcatgggcaaaatgcacctggcatgccgtatatcctctcatggctcctgcagaagggttattggtatacacacgccttgccaggaaatccacggaattcatcttgtaagggaagttggcccacaatgtggactgggcgcaggccgcaacaccggacccgccgtaaggcccgccgtccagcacatggtagcatttctttgccagcagcttaccgtctgtcccaaaggcagtgtcaatatgcatgtaaatggggtggcggttgcgcgtggtctggaatacttcttcgcgggacagaatcatgcgtaccgggcgtccggtcatctccgccatcttggcagcgcaaaggccaaaggaataggaatccagcttgccgccgaaaccgccgcccacaagaggcttgattacccgcacctggttctctccaacgccaaggcagcgggcataccagaactggtccacaaaggacatctgggtggacatccagatggtgtaggtcccattcctgtaggtagccaccgcaccgtggggctccatggccgcatgtaccatacggtgggtcttgtaatccctgtgctgcacataggatgcgcggtcaaattcctcatcaatatccgtgcccgccttcatcacggactgcatgccgatattgtgtatgcctttgccctcccagtttacctcgggggcattctcctccattgcctcaaaggggtcaaacacccccggaagcacctggtactctaccttaatcagatccgcggcccgctgggcggtttcctcatccacggctgccacggctgccacatcgtcaccaacctggcgcaccttctcagaacacaatacttccttgtccgcgaactcagctgcaaattctccatttcccaccagggacttccactcaaagtccctggcagtgaggatgcactttacacctggaagcttctctgcctcgctggtgtcaatggacaggatttttgcagatgcataagggcttctgaccatttttccggtaagcatatccggaaacatgatgtcacccacatactggccgtgtcctgttaccttgtcttcagcgtcaatcctgacataattgttctcgccggtcagacggtaaaattccggttttttaaaataatgtttgtcacagtctttatgcat

SEQ ID NO: 13 - DNA, 867 bp, Clostridium asparagiforme
ctataagctttccatggcctgtttaatggcacgtttggtaaatacacgaatcatatccttccggtattcggccgacgcacggatatcggaaattggatgacaggaattcattgcctcttctgacgccctcacaatgacttcgtcggtaagggccttcccgatcagggcttcctccgccctgggagcgcggatcggagttgcagccactgcgcccagagcaatcttcgcatctgtgcagataccgacctccaccctgattttaaccgcaacgccgataatcgccagatccatggcttttctgacagcgtgctttatgtacgcggctctctcattctctgccagaggcgggatcacaatacctgttacgatctctcccggctccagggatgtttttttcactcccaggaaaaagtcgtctattttgatgacccggtccttgttggggccctgaaccaggatcttcgcgccctgtgccaatagatttggcgccgtgtcgcaggacggggatgcgttgcagatatttcccgccatggtacccttggcgcgaatctgggtggatgccaccaccttggccgcatgtgcgatggccggatttttctcttttacaagaggagaggtctcgatggcgcgcagggtggtgagcgctccgatcttaagcccttccttctcgtcatactccagatcatccagacccggaatcttctttaggtcaatgatatactccggcgcaataaccttatccttcataggcggaatcaggtctgttgcgcctgccatgacttttgccgtgcttccaagctcgaggagcagattgcacgcctcaccgatggtcttaggggccagatactcaaattgaggtaataccat

SEQ ID NO: 14 - DNA, 492 bp, Clostridium asparagiforme
ttatgcattctctgattcctcctcccagttcatttcgtccgcagctgcctggatcgcttccacgatcttggcataaccggtacagcggcacaggttgccctcgatggcttcccggatctccagctctgtgggatgcctgttcacatctaacaacgccttggcggacataatcatgccaggggtacagtagccgcactgcatggcccatttttcaatgaactgcttctgaatcggatgaagcatcccttctttggcaacgccctccacagtcaaaatctcatggccgtcacattccacagccagagtacaacaggagttgaccggctttccgtccagcataacggtacacgcgccgcactccccttcctcgcatcccttcttcgtgccggtcagaaacatctggtcacgaaggaaatccagaagcgtcagattatctttcacaatggcatcaaccggatctccgttgataattaaacttatactatgtttcat

SEQ ID NO: 15 - DNA, 2364 bp, Clostridium asparagiforme
ttatttagagttcctgtcatctttcattccgtgcagcgctctccagatatgctccggatccaggggcagttcggtaaaataaactccggtcgccatgttaaccgcgttggcgatagccggcgccaccggcgctgcggagccttcgccggcttccttggcgcccagcggtccttcctcgtccggcgtaaagtcgtagaacgtgcgcatcttgggcatatccagagcggtgggcagacggtaatcgcggaagttgggattgaggatcttaccttccttcgttacattgtgttcgtaaaccgcgtatccgaggcccattccgatggagccctccagctggccttctacagccctcttattcagtgcgcggccgcaatcatgggcaaatacgaactcgtcgatatccagcacgccggtctcctcgtccacggtcaggtgggccgcgccagtggagaagctatacgcaggagcgtagttggtggtattggttccgttgtactgggagttgtcggtgcggtggtagtaggaacccacaccgatcagctcatccccgcccttgacggtcatgtacttgaacatagcgtctccgatgggcatttgaagttgggcgttctccctgctgatcaccttgccgtccaggcactccagggtttcgggcatcacgccccacatgggagcaatcacctcaaacagctgtcgtttggcatccacggcagcgcggcgggccgcattgcctgcaaggaatgtgacgcggcttccatatgaaccggaatcccagggtgtcaggaaggtatcggacataaatgtctttaccatgttcatgggcagacccagttcctctgccacgatagcggtcataaccgtgtcggagccctggccgatatcatgagaaccgatgtacagggtcgccataccacgtttattcatacgaagggtgacgcatgcggagctctggttgggagcttccagcaccgcgaagccggttcctgacacaaacccggttccggcaaagccaatgccttcgcccttcttcatcttatccttcttctcattccagccaatttccctggctgccgtatccagcgtctccttgtaggcacaactggtgatggccagtccggcgggcgccacatagcccgggtctgctgcgctgatcttgcggaattccaccgggtccatgcccagctgatccgcagcgaactgcatgttcaggtcatgggcaaaatgcacctggcatgcggtatatcctctcatggctccggccgacgggttgttggtatacacacgccttgccaggaaatccacggaattcatcttataagggaagttagcccacagcgtagactgcgcgcacgccgccacaccagaaccgccgtaagggccgccgtccagcacgtgatagcatttcttggccagaagccttccgtccgcgccgaatgcggtatcaatgtgcatatagatcggatggcggttacgtgtggtctgaaacacttcctctcgggacagaatcatgcgcactgggcgtcctgtaatctcggacatcttggccgcgcacaggccgaaggagtaggaatccagcttaccgccaaatcctccgcctactaacggcttaatcacacgaacctggttctctcccacccccaaacagcgcgcataccagaactgatccacaaaggacatctgtgtggacatccagatcgtataagtaccatttcggtaggttgctacagctccgtgcggctccatggcagcatggaccatacggtgtgtcttataatccctgtgctgcacataagatgcgctgtcaaattcctggtcgatatccgtgcccgccttcatcacggactgcataccgatgttatggatgcccttgccctcccagttcacctcgggagcgtcgtcctccatggcttcaaacggatcgaacacgccgggaagcacttcgtactccacctttatgaggtccactgccctctgggctgtctcttcatccaccgccgcgacggcagcaatatcgtcgccaacctggcgtaccttttccgagcagagcacttccttatccgcaaactctgccgcgaactcaccgtttcccaccagggatttccactcaaaatccttcgctgtcaggatacactttaccccgggcagcttctccgccgcacttgtgtcgatggaaatgattctggcggaagcatatggacttctgaccattttcccggtcagcatatcagggaacataatatcgcccacatactggccgtgtcccgttactttgtcttccgcgtcaattctcacataattattaccgccggtgagacggtagaattccggtttcttaaaataatgcttgtcacaatctttatgcat

SEQ ID NO: 16 - DNA, 867 bp, Clostridium citroniae
atggtattacctcaattcgagtatctggctcctaagaccataggggaggcatgtaatctgctccttgagcttggaagcccggcaaaagtcatggcaggagcaacggatctgatcccgcccatgaaagacaaagcgatttcgccggagtatctcattgatctgaagaagatcccggatctggattatctggaatatgatgaaaaggaagggttaaagatcggcgcactgacaaccctgcgcaccattgagacctcacctttggtaaaagaaaagaacccggctgtggcccatgccgccaaggtagtggcttccacacagatcagggcaaagggcaccatggcgggaaatatctgcaatgcttccccctcctgtgacacggcgcccaaccttttggcccagggggcaaagatcttagtacaggggcccaacaaggaccgtatcattcaggcggaggattttttcctgggtgtaaagaaaacctcactggaaccgggggagatcgtaacagggattgtgatcccgcccctggcagagaatgaaagggctgcttacataaaacacgctgtgagaaaagccatggatctggccattatcggtgttgcggttaagatcaaggtggaggacggcatatgcacggatgtgcatatcgccctgggcgcagtggcagccacacctatccgcgcccccaaggcagaggaggctctgatcggcaaggcccttaccgatgaggttattgtaaaggcatcggaggaggccatggattcctgtcatcctatttctgatatccgtgcatcagccgaataccgcaaggatatgatccgtgtatttaccaagcgtgccgtcaggcaggccatggaatgtttatag

SEQ ID NO: 17 - DNA, 492 bp, Clostridium citroniae
atgaagcatagtataagtttaaccgttaacggagactgcgttgacgccgttgtgaaagataacctgacactgctggatttccttcgtgaccagctgtttttaaccggtacaaaaaaaggatgtgaggaaggggaatgcggcgcatgtacggttatgctggacgggaaaccggtcaattcctgctgtaccctggccgtggagtgcgatggccatgacattatcaccgtggaaggcattgcagagaacggaatgctccaccccatccagaagcagtttattgaaaagtgggccatgcagtgcggttactgtaccccgggcatgatcatgtccgccaaggcattgctggatgttaaccgtcatcccacggaactggagatccgggaagccattgagggcaacctgtgccgatgtaccggctatgccaagatcgtggaggcgatccaggctgccgccgcacaaatgaactgggaggaggaatcagagaatgcataa

SEQ ID NO: 18 - DNA, 2364 bp, Clostridium citroniae
atgcataaagactgtgacaaacattattttaaaaagccggaattctaccgtctcaccggtgagaatcattatgtgaggattgacgcggaagacaaagtgacgggccacggccagtatgtgggcgacatcatgtttccggatatgctgaccggcaagatggtgagaagcccctatgcctcggccaggatcctttccattgacaccagcgaagccgaaaagctgccgggtgtaaaatgtatcctcacggcaaaggactttgagtggaagtccttggtgggcaacggagagtttgccgctgaatttgcagacaaggaagtactttgctccgagaaggtccgccaggtaggggatgatgtggcggcagtggcggcagtggatgaggagacggcccagagggcggttgacctgatcaaggtggagtatgaggtgcttccgggtgtatttgatccctttgaggccatggaggaaggcgctcccgaggtcaactgggagggcaaaggacttcacaatatcggtatgcagtccgtgatgaaggcgggcacggacattgaccaggagtttgacaacgcgggctatgtacagcacagggattacaagacccaccgtatggtccatgcggccatggagccccacggcgcggtggccacgttcagaaacggcacctataccatctggatgtccacgcagatgtcctatgtggaccagttctggtatgcccgctgcctgggcgtgggggagaaccaggtgcgcgtgatcaagccgctggtaggcggcggattcggaggaaagctggattcctattcctttggactctgcgctgccaagatgtcggaactgaccggacggcctgtgcgtatgatcctgtcccgtgaggaggtattccagaccacacgtaaccgccatcccatctatatgcacattgacactgcctttggcgcggacggaaagctgctggcgaaaaaatgctaccatgtgctggacggcggcccctacggcggttccggtgttgcggcctgcgcccagtccacactgtgggccaacttcccatataagatgaattccgtggatttcctggcaagacgtgtgtacaccaacaacccgtcagccggtgccatgaggggctacacggcgtgccaggtgcattttgcccatgacctgaatatgcagtttgcagcggaccagatggggatcgacccggttgagttccgtaagatgagcgcggcggaccctggatatgtggctcccgcggggctggctattaccagctgcgcttacaaagagactttggatacggctgccagggaaattggctggtatgataaaaaggatcagatgaaaaagggcgagggcattggctttgccggaaccggatttgtatccggaaccggattcgcggtgctggaagctccgaaccagagttctgcgtgcgtgacactgcgcatgaacaagcggggcatggcaactctttacattggttcccatgatatcggccagggctcagatacggtcatgacagcgatcgtggcagaggaactgggccttcccatggatatggtaaagacattcatgtccgataccttcctgacaccctgggattccggttcttacggaagccgtgttaccttccttgcgggaaatgctgcccgccgcgctgccgtggatgcaaagcgccagctgtttgaggtgatcgctcccatgtggggtgtgatgcctgaaacactggagtgtctggacggcaaggtgatcagcaaagagaacgcagagcttcagatgcccattggggacgccatgtttaagtatatgaccgttaagggaggcgatgagctggtgggtatcggctcatattaccaccgcaccgacaattcccagtacaatggtaccaataccaccaactacgcgccggcttacagtttttccacaggagcggcccatctgaccgtggatgaggagacaggcgtgctggatatcgatgagtttgtatttgcccatgactgcggccgcgccctgaacaagagggctgtggaaggccagctggagggttccatcggcatgggacttggatatgcggtctacgagcacaacgtgaccaaggagggcaagatattaaatcctaatttccgtgattaccgtctgccaaccgcccttgacatgccgaagatgcgtaccttttacgattttacaccggatgaggaaggacctctgggtgcaaaggaagcaggggaaggctcggcagcgccggtggcgcctgccattgccaatgcggtcaacatggctaccggtgtatattttacggagcttccactggatcccgaacatatctggagagcgctccatggacttaaggatgacaggaattccaaataa

SEQ ID NO: 19 - DNA, 870 bp, Artificial Sequence
  CbUroC1_opt
atggtcctcccgcagttcgagtacctcgccccgaagaccatcggcgaggcctgcaacctcttcctcgaactcggctcgaccgcccgcgtcatggcaggtgcaaccgacctcatcccgccgatgaaggacaaagtcatctcgccggagtacatcatcgacctcaagaagatcccgggcctcgactacctcgaatacgacgaccgcgaaggcctcaagatcggcgccctcaccaccctccgcaccatcgaaacctcgccgctcgtcaaggaaaagaacccggccgtcgcccacgccgccaaggtcgtcgcatcgacccaaatccgaaccaagggcaccatggccggcaacatctgcaacgcctcgccgtcgtgcgacaccgcaccgaacctcctcgcacagggtgcaaagatcctcgtccagggtccgaacaaggaccgcgtcatccagatcgaggacttcttcctcggcgtcaagaagacctcgctcgagccgggcgaaatcgtcaccggcatcgtcatcccgccgctcgccgaaaacgaacgcgcagcctacatcaagcacgccgtccgcaaggccatggacctcgccatcatcggcgtcgccgtcaagatcaaggtcgaagacggcgtctgcaccgacgcccgcatcgcactcggtgcagtcgcagcaaccccggtccgagcaccgggtgcagaagaagcactcatcggcaaggaactcaccgacgaggtcatcgtcaaggcctcggaggaggccatgaactcgtgccacccgatctcggacatccgcgcctcggccgaataccgcaaggacatgatccgcgtcttcaccaagcgcgccatcaagcaggccatggagtgctacaactga

SEQ ID NO: 20 - DNA, 492 bp, Artificial Sequence
  CbUroC2_opt
atgaagcactcgatctcgctcatcatcaacggcgacccggtcgacgccatcgtcaaggacaacctcaccctcctcgacttcctccgcgaccagctcttcctcaccggcaccaagaagggctgcgaagagggcgaatgcggcgcctgcaccgtcatgctcgacggaaagccggtcaactcgtgctgcaccctcgccgtcgaatgcgacggccacgaaatcatcaccgtcgaaggcatcgcccgcgaaggcatgctccacccgatccagaagcagttcatcgagaagtgggccatgcagtgcggctactgcaccccgggcatgatcatgtcggccaaggccctcctcgacgtcaacaagcacccgaccgaactcgaaatccgcgaagccatcgaaggcaacctctgccgctgcaccggctacgccaagatcgtcgaagccatccaggcagccgccgcccagatgaactgggaagaagaggccaagaacgcctga

SEQ ID NO: 21 - DNA, 2364 bp, Artificial Sequence
  CbUroC3_opt
atgcacaaggactgcgacaagcactacttcaagaagccggagttctaccgcctcaccggcgagaacaactacgtccgcatcgacgccgaagacaaggtcaccggccacggccagtacgtcggcgacatcatgttcccggacatgctcaccggcaagatggtccgctcgccgtacgcatcggccaagatcctctcgatcgacacctcggaggccgagaagctcccgggcgtcaagtgcatcctcaccgcccgcgacttcgagtggaagtcgctcgtcggcaacggcgagttcgcggccgaattcgccgacaaggaagtcctctgctcggaaaaggtccgccaggtcggcgacgacgtcgcagcagtcgcagcagtcgacgaagaaaccgcccaacgcgcagccgatctcatcaaggtcgaataccaggtcctcccgggcgtcttcgacccgttcgaggccatggaggagaacgccccggaggtcaactgggagggcaagggcatccacaacatcggcatgcagtcggtcatgaaggccggcaccgacatcgacgaagaattcgaccgcgcctcgtacgtccagcaccgcgactacaagacccaccgcatggtccacgccgccatggaaccgcacggtgcagtcgcaacctaccgcaacggtacctacaccatctggatgtcgacccagatgtcgttcgtcgaccagttctggtacgcccgctgcctcggtgtcggcgaaaaccaggtccgcgtcatcaagccgctcgtcggcggtggcttcggcggtaagctcgactcgtactcgttcggactctgcgccgccaagatggccgaaatgaccggacgcccggtccgcatgatcctctcgcgcgaggaagtcttccagaccacccgcaaccgccacccgatctacatgcacatcgacaccgccttcggcaccgacggcaagctcctcgccaagaagtgctaccacgtcctcgacggcggcccgtacggtggatcgggtgtcgcagcatgcgcacaatcgaccctctgggccaacttcccgtacaagatgaactcggtcgacttcctcgcccgccgcgtctacaccaacaacccgtcggcaggagcaatgcgcggctacaccgcatgccaggtccacttcgcccacgacctcaacatgcagttcgccgccgaccagatgggcatcgacccggtcgaattccgcaagatctcggccgccgacccgggttacgtcgcaccggcaggactcgcaatcacctcgtgcgcatacaaggaaaccctcgacaccgccgccaaggagatcggctggtacgagaagaaggacaagctcaagaagggcgaaggcatcggcttcgccggcaccggtttcgtctcgggaaccggattcgccgtcctcgaagccccgaaccaatcgtcggcctgcgtcaccctccgcatgaacaagcgcggcatggccaccctctacatcggctcgcacgacatcggccagggctcggacaccgtcatgaccgccatcgtcgcagaagaactcggcctcccgatggacatggtcaagaccttcatgtcggacaccttcctcaccccgtgggactcgggctcgtacggatcgcgcgtcaccttcctcgcaggaaacgcagcccgccgcgcagcggtggatgcaaagcgccaactcttcgaagtcatcgccccgatgtggggcgtcatgccggaaaccctcgaatgcctcgacggcaaggtcatctcgaaggagaaggccgagtaccagatgtcgatcggcgacgccatgttcaagtacatgaccgtcaagggcggcgacgaactcatcggcgtcggctcgtactaccaccgcaccgacaactcgcagtacaacggcaacaacaccaccaactacgccccggcctactcgttctcgaccggagcagcacacctcaccgtcgacgaggagacgggagtcctcgacatcgacgagttcgtcttcgcccacgactgcggccgcgcactcaacaagcgcgcagtcgaaggtcagctcgaaggctcgatcggcatgggcctcggttacgccgtctacgagcacaacgtcacccgcgagggcaagatcctcaacccgaacttccgcgactaccgcctcccgaccgcactcgacatgccgaagatgcgcaccttctacgacttcaccccggacgaagaaggcccgctcggagccaaggaagcaggtgaaggatcggccgcaccggtcgcaccggcaatcgcaaacgcagtcaacatggcaaccggcgtctacttcaccgaactcccgctcgacccggaacacatctggcgcgcactccacggtatgaaggacgaccgcaactcgaagtga

SEQ ID NO: 22 - DNA, 3753 bp, Artificial Sequence
  CbUroC123_opt
atggtcctcccgcagttcgagtacctcgccccgaagaccatcggcgaggcctgcaacctcttcctcgaactcggctcgaccgcccgcgtcatggcaggtgcaaccgacctcatcccgccgatgaaggacaaagtcatctcgccggagtacatcatcgacctcaagaagatcccgggcctcgactacctcgaatacgacgaccgcgaaggcctcaagatcggcgccctcaccaccctccgcaccatcgaaacctcgccgctcgtcaaggaaaagaacccggccgtcgcccacgccgccaaggtcgtcgcatcgacccaaatccgaaccaagggcaccatggccggcaacatctgcaacgcctcgccgtcgtgcgacaccgcaccgaacctcctcgcacagggtgcaaagatcctcgtccagggtccgaacaaggaccgcgtcatccagatcgaggacttcttcctcggcgtcaagaagacctcgctcgagccgggcgaaatcgtcaccggcatcgtcatcccgccgctcgccgaaaacgaacgcgcagcctacatcaagcacgccgtccgcaaggccatggacctcgccatcatcggcgtcgccgtcaagatcaaggtcgaagacggcgtctgcaccgacgcccgcatcgcactcggtgcagtcgcagcaaccccggtccgagcaccgggtgcagaagaagcactcatcggcaaggaactcaccgacgaggtcatcgtcaaggcctcggaggaggccatgaactcgtgccacccgatctcggacatccgcgcctcggccgaataccgcaaggacatgatccgcgtcttcaccaagcgcgccatcaagcaggccatggagtgctacaactgagaaggagacaggaatgaagcactcgatctcgctcatcatcaacggcgacccggtcgacgccatcgtcaaggacaacctcaccctcctcgacttcctccgcgaccagctcttcctcaccggcaccaagaagggctgcgaagagggcgaatgcggcgcctgcaccgtcatgctcgacggaaagccggtcaactcgtgctgcaccctcgccgtcgaatgcgacggccacgaaatcatcaccgtcgaaggcatcgcccgcgaaggcatgctccacccgatccagaagcagttcatcgagaagtgggccatgcagtgcggctactgcaccccgggcatgatcatgtcggccaaggccctcctcgacgtcaacaagcacccgaccgaactcgaaatccgcgaagccatcgaaggcaacctctgccgctgcaccggctacgccaagatcgtcgaagccatccaggcagccgccgcccagatgaactgggaagaagaggccaagaacgcctgagaaggagtctcgcaatgcacaaggactgcgacaagcactacttcaagaagccggagttctaccgcctcaccggcgagaacaactacgtccgcatcgacgccgaagacaaggtcaccggccacggccagtacgtcggcgacatcatgttcccggacatgctcaccggcaagatggtccgctcgccgtacgcatcggccaagatcctctcgatcgacacctcggaggccgagaagctcccgggcgtcaagtgcatcctcaccgcccgcgacttcgagtggaagtcgctcgtcggcaacggcgagttcgcggccgaattcgccgacaaggaagtcctctgctcggaaaaggtccgccaggtcggcgacgacgtcgcagcagtcgcagcagtcgacgaagaaaccgcccaacgcgcagccgatctcatcaaggtcgaataccaggtcctcccgggcgtcttcgacccgttcgaggccatggaggagaacgccccggaggtcaactgggagggcaagggcatccacaacatcggcatgcagtcggtcatgaaggccggcaccgacatcgacgaagaattcgaccgcgcctcgtacgtccagcaccgcgactacaagacccaccgcatggtccacgccgccatggaaccgcacggtgcagtcgcaacctaccgcaacggtacctacaccatctggatgtcgacccagatgtcgttcgtcgaccagttctggtacgcccgctgcctcggtgtcggcgaaaaccaggtccgcgtcatcaagccgctcgtcggcggtggcttcggcggtaagctcgactcgtactcgttcggactctgcgccgccaagatggccgaaatgaccggacgcccggtccgcatgatcctctcgcgcgaggaagtcttccagaccacccgcaaccgccacccgatctacatgcacatcgacaccgccttcggcaccgacggcaagctcctcgccaagaagtgctaccacgtcctcgacggcggcccgtacggtggatcgggtgtcgcagcatgcgcacaatcgaccctctgggccaacttcccgtacaagatgaactcggtcgacttcctcgcccgccgcgtctacaccaacaacccgtcggcaggagcaatgcgcggctacaccgcatgccaggtccacttcgcccacgacctcaacatgcagttcgccgccgaccagatgggcatcgacccggtcgaattccgcaagatctcggccgccgacccgggttacgtcgcaccggcaggactcgcaatcacctcgtgcgcatacaaggaaaccctcgacaccgccgccaaggagatcggctggtacgagaagaaggacaagctcaagaagggcgaaggcatcggcttcgccggcaccggtttcgtctcgggaaccggattcgccgtcctcgaagccccgaaccaatcgtcggcctgcgtcaccctccgcatgaacaagcgcggcatggccaccctctacatcggctcgcacgacatcggccagggctcggacaccgtcatgaccgccatcgtcgcagaagaactcggcctcccgatggacatggtcaagaccttcatgtcggacaccttcctcaccccgtgggactcgggctcgtacggatcgcgcgtcaccttcctcgcaggaaacgcagcccgccgcgcagcggtggatgcaaagcgccaactcttcgaagtcatcgccccgatgtggggcgtcatgccggaaaccctcgaatgcctcgacggcaaggtcatctcgaaggagaaggccgagtaccagatgtcgatcggcgacgccatgttcaagtacatgaccgtcaagggcggcgacgaactcatcggcgtcggctcgtactaccaccgcaccgacaactcgcagtacaacggcaacaacaccaccaactacgccccggcctactcgttctcgaccggagcagcacacctcaccgtcgacgaggagacgggagtcctcgacatcgacgagttcgtcttcgcccacgactgcggccgcgcactcaacaagcgcgcagtcgaaggtcagctcgaaggctcgatcggcatgggcctcggttacgccgtctacgagcacaacgtcacccgcgagggcaagatcctcaacccgaacttccgcgactaccgcctcccgaccgcactcgacatgccgaagatgcgcaccttctacgacttcaccccggacgaagaaggcccgctcggagccaaggaagcaggtgaaggatcggccgcaccggtcgcaccggcaatcgcaaacgcagtcaacatggcaaccggcgtctacttcaccgaactcccgctcgacccggaacacatctggcgcgcactccacggtatgaaggacgaccgcaactcgaagtga

SEQ ID NO: 23 - DNA, 36 bp, Artificial Sequence
  SYN6606 F01
taagaaggagatatacatggtcctcccgcagttcga

SEQ ID NO: 24 - DNA, 36 bp, Artificial Sequence
  SYN6606 R02
gtgatggtggcccatgtcacttcgagttgcggtcgt